European Patent Application EP 4 327 832 A1, published February 28, 2024. Title: ANTI-SEZ6 ANTIBODY DRUG CONJUGATES. Applicant: AbbVie Biotherapeutics, Inc. Application US. The sequence listing filed with the application follows.

SEQUENCE LISTING (12 sequences)

SEQ ID NO: 1 - protein, 115 aa, synthetic construct
EVQLVQSGAEVKKPGESLKISCKGSGYSFTSSWINWVRQMPGKGLEWMGRIYPGEGDTNYNGNFEGQVTISADKSISTAYLQWSSLKASDTAMYYCTRGLVMDYWGQGTLVTVSS

SEQ ID NO: 2 - protein, 111 aa, synthetic construct
EIVLTQSPATLSLSPGERATLSCRASQSVDYNGISYMHWYQQKPGQAPRLLIYAASNVQSGIPARFSGSGSGTDFTLTISSLEPEDFAVYYCQQSIEDPPTFGGGTKVEIK

SEQ ID NO: 3 - protein, 10 aa, synthetic construct
GYSFTSSWIN

SEQ ID NO: 4 - protein, 17 aa, synthetic construct
RIYPGEGDTNYNGNFEG

SEQ ID NO: 5 - protein, 6 aa, synthetic construct
GLVMDY

SEQ ID NO: 6 - protein, 15 aa, synthetic construct
RASQSVDYNGISYMH

SEQ ID NO: 7 - protein, 7 aa, synthetic construct
AASNVQS

SEQ ID NO: 8 - protein, 9 aa, synthetic construct
QQSIEDPPT

SEQ ID NO: 9 - protein, 444 aa, synthetic construct
EVQLVQSGAEVKKPGESLKISCKGSGYSFTSSWINWVRQMPGKGLEWMGRIYPGEGDTNYNGNFEGQVTISADKSISTAYLQWSSLKASDTAMYYCTRGLVMDYWGQGTLVTVSSASTKGPSVFPLAPSSKSTSGGTAALGCLVKDYFPEPVTVSWNSGALTSGVHTFPAVLQSSGLYSLSSVVTVPSSSLGTQTYICNVNHKPSNTKVDKKVEPKSSDKTHTCPPCPAPELLGGPSVFLFPPKPKDTLMISRTPEVTCVVVDVSHEDPEVKFNWYVDGVEVHNAKTKPREEQYNSTYRVVSVLTVLHQDWLNGKEYKCKVSNKALPAPIEKTISKAKGQPREPQVYTLPPSRDELTKNQVSLTCLVKGFYPSDIAVEWESNGQPENNYKTTPPVLDSDGSFFLYSKLTVDKSRWQQGNVFSCSVMHEALHNHYTQKSLSLSPG

SEQ ID NO: 10 - protein, 218 aa, synthetic construct
EIVLTQSPATLSLSPGERATLSCRASQSVDYNGISYMHWYQQKPGQAPRLLIYAASNVQSGIPARFSGSGSGTDFTLTISSLEPEDFAVYYCQQSIEDPPTFGGGTKVEIKRTVAAPSVFIFPPSDEQLKSGTASVVCLLNNFYPREAKVQWKVDNALQSGNSQESVTEQDSKDSTYSLSSTLTLSKADYEKHKVYACEVTHQGLSSPVTKSFNRGEC

SEQ ID NO: 11 - DNA, 1998 bp, synthetic construct
  source 1..1998: mol_type = other DNA
atggaatggtcctgggtgttcctgttcttcctgtccgtgaccaccggtgtgcactccgaagtccaactcgtccaatccggtgccgaagtgaaaaagcctggggaatccctgaagatcagctgcaagggatccggttactcgttcacctcctcctggattaactgggtccggcagatgcccggaaagggactggagtggatgggcagaatctatccgggcgaaggggacactaattacaacggaaacttcgagggccaggtcaccatttcggccgataagagcatctcaaccgcgtacttgcagtggtcaagcctgaaggcttccgacaccgccatgtactactgtactcgcggccttgtgatggactactggggacagggaactctcgtgaccgtgtcgtccgcctctaccaagggcccttccgtgttccctctggccccctcgagcaagagcacctctgggggcacagcggccctgggctgcctggtcaaggactacttccccgagccggtgacggtgtcgtggaactcaggcgccctgaccagcggcgtgcacaccttcccggctgtcctacagtcctcaggactctactccctcagcagcgtggtgaccgtgccctccagcagcttgggcacccagacctacatctgcaacgtgaatcacaagcccagcaacaccaaggtggacaagaaagttggtgagaggccagcacagggagggagggtgtctgctggaagccaggctcagcgctcctgcctggacgcatcccggctatgcagccccagtccagggcagcaaggcaggccccgtctgcctcttcacccggaggcctctgcccgccccactcatgctcagggagagggtcttctggctttttccccaggctctgggcaggcacaggctaggtgcccctaacccaggccctgcacacaaaggggcaggtgctgggctcagacctgccaagagccatatccgggaggaccctgcccctgacctaagcccaccccaaaggccaaactctccactccctcagctcggacaccttctctcctcccagattccagtaactcccaatcttctctctgcagagcccaaatctagtgacaaaactcacacatgcccaccgtgcccaggtaagccagcccaggcctcgccctccagctcaaggcgggacaggtgccctagagtagcctgcatccagggacaggccccagccgggtgctgacacgtccacctccatctcttcctcagcacctgaactcctggggggaccgtcagtcttcctcttccccccaaaacccaaggacaccctcatgatctcccggacccctgaggtcacatgcgtggtggtggacgtgagccacgaagaccctgaggtcaagttcaactggtacgtggacggcgtggaggtgcataatgccaagacaaagccgcgggaggagcagtacaacagcacgtaccgtgtggtcagcgtcctcaccgtcctgcaccaggactggctgaatggcaaggagtacaagtgcaaggtctccaacaaagccctcccagcccccatcgagaaaaccatctccaaagccaaaggtgggacccgtggggtgcgagggccacatggacagaggccggctcggcccaccctctgccctgagagtgaccgctgtaccaacctctgtccctacagggcagccccgagaaccacaggtgtacaccctgcccccatcccgggatgagctgaccaagaaccaggtcagcctgacctgcctggtcaaaggcttctatcccagcgacatcgccgtggagtgggagagcaatgggcagccggagaacaactacaagaccacgcctcccgtgctggactccgacggctccttcttcctctacagcaagctcaccgtggacaagagcaggtggcagcaggggaacgtcttctcatgctccgtgatgcatgaggctctgcacaaccactacacgcagaagagcctctccctgtctccgggttga

SEQ ID NO: 12 - DNA, 717 bp, synthetic construct
  source 1..717: mol_type = other DNA
atggagacagacacactcctgctatgggtactgctgctctgggttcccgggtccactggtgaaatcgtgttgacccagtcccccgctaccctgtcactgagccccggagaacgcgcgactctgtcctgccgggcatcccagtccgtggactacaacggaatctcctacatgcactggtatcagcaaaagccaggccaagccccgagactgctcatctacgccgcctcgaacgtgcagagcggtattccggcgcggttctccggctcgggcagcggaaccgattttaccctcactatctcgtcacttgaacctgaggacttcgccgtgtactactgccagcagtccattgaggacccgcctactttcggggggggaaccaaagtcgagatcaagcggactgtggctgcaccaagtgtcttcatcttcccgccatctgatgagcagttgaaatctggaactgcctctgttgtgtgcctgctgaataacttctatcccagagaggccaaagtacagtggaaggtggataacgccctccaatcgggtaactcccaggagagtgtcacagagcaggacagcaaggacagcacctacagcctcagcagcaccctgacgctgagcaaagcagactacgagaaacacaaagtctacgcctgcgaagtcacccatcagggcctgagctcgcccgtcacaaagagcttcaacaggggagagtgttga